European Patent Application EP 4 134 454 A1, published February 15, 2023. Title: Reagent Combination and Kit for Detecting Liver Cancers, and Use Thereof. Applicant: SANSURE BIOTECH INC. Application EP21893921.3. The sequence listing filed with the application follows.

SEQUENCE LISTING (6 sequences)

SEQ ID NO: 1 - DNA, 353 bp, Homo sapiens
ccgtgtcaccactctccgaaagccggcggagatcccccagaacccggcccagctaggggagccccaggcagggccggcattacctggtggggaaggctagccccggcatctctggcgattgtttccgtcgcagagccgcacctctccctgcccaaccgggtacccacaaggcccctgctccaccggctccgctcgattcagctgggctgggctcctggcagctcagccgccagctcccgaggtgcagcacgctcgcgctctcgcagggcggcagcgaaggcgccgcgtcggggttggcgaaacagaaggggcgggggaagaaaggagggaaggaggcgggaggaagccgcgcg

SEQ ID NO: 2 - DNA, 172 bp, Homo sapiens
cgattttgctccacgcctgccggccagagcctcccggcgtttcttccgccccagcggagtgcgctggggcgcgccagggctaggcccgccggaggagcgcgtccccagccttccgcgcacagagccgcatcccgccccgccctgcgctggactggttcaagcttccgcctcg

SEQ ID NO: 3 - DNA, 216 bp, Homo sapiens
cgccccactcacccttcgctctaccggcggcggcgggaacccacccccgggagcgagaacaatgcccggccgcacgcgcgccggaagtgggagagtgcccctctaggagcccggaggaccgcagctctgtggcaggcgcgggtcgtgtctcgcaggaggggcgcgggtccggctcagacctggcgggggcatcgcagagtacaagcggttgacgcg

SEQ ID NO: 4 - DNA, 81 bp, Homo sapiens
cgcagccgccacccctgggcccccagcggacgagctgtacgcggcgctggaggactatcaccctgccgagctgtaccgcgc

SEQ ID NO: 5 - DNA, 341 bp, Homo sapiens
cggtcccgaccccgggaccccctgccgcagccgccacccctgggcccccagcggacgagctgtacgcggcgctggaggactatcaccctgccgagctgtaccgcgcgctcgccgtgtccgggggcaccctgccccgccgaaaggtgcgtcccccgcccgccttcaggatctgctcagcccctctccgactccctacagggcctgctgactccgcagtgccctctcctcggcgtccgcggagtcccccaccttcttccccggcccgctgggtgcctcgactccccgcgttccccgctgctgcgaaggccgtggccctcgcctgcacaccgcgcccaggctcg

SEQ ID NO: 6 - DNA, 232 bp, Homo sapiens
cgacccagtgttaacagggaatggttattctgtacgggcatctgaactgaaaagtgagaagagcgaactttgcctcctcggccccttctctgtgcctgtggcttatgcgtgtgcccctctcctctttgtcactgcttcccttgccctggatgtggttggtgcactggggtcaccttagaccacaggaaatgtctggttaacacacgaagagatggaaacgctcgcagccacg